European Patent Application EP 4 206 226 A1, published July 5, 2023. Title: Hexameric anti-VEGF antibody, and compositions comprising the same. Applicant: Medytox Inc. The sequence listing filed with the application follows.

SEQUENCE LISTING (76 sequences)

SEQ ID NO: 1 - DNA, 38 bp, Artificial Sequence
  primer
gggcccaggcggccgagctcgtgmtgacccagactcca

SEQ ID NO: 2 - DNA, 38 bp, Artificial Sequence
  primer
gggcccaggcggccgagctcgatmtgacccagactcca

SEQ ID NO: 3 - DNA, 38 bp, Artificial Sequence
  primer
gggcccaggcggccgagctcgtgatgacccagactgaa

SEQ ID NO: 4 - DNA, 36 bp, Artificial Sequence
  primer
tctagaggaaccacctaggatctccagctcggtccc

SEQ ID NO: 5 - DNA, 36 bp, Artificial Sequence
  primer
tctagaggaaccacctttgatttccacattggtgcc

SEQ ID NO: 6 - DNA, 36 bp, Artificial Sequence
  primer
tctagaggaaccacctttgacsaccacctcggtccc

SEQ ID NO: 7 - DNA, 40 bp, Artificial Sequence
  primer
gggcccaggcggccgagctcgtgctgactcagtcgccctc

SEQ ID NO: 8 - DNA, 36 bp, Artificial Sequence
  primer
tctagaggaaccacctgtgacggtcagctgggtccc

SEQ ID NO: 9 - DNA, 21 bp, Artificial Sequence
  primer
cagtcggtggaggagtccrgg

SEQ ID NO: 10 - DNA, 21 bp, Artificial Sequence
  primer
cagtcggtgaaggagtccgag

SEQ ID NO: 11 - DNA, 21 bp, Artificial Sequence
  primer
cagtcgytggaggagtccggg

SEQ ID NO: 12 - DNA, 23 bp, Artificial Sequence
  primer
cagsagcagctgrtggagtccgg

SEQ ID NO: 13 - DNA, 37 bp, Artificial Sequence
  primer
actggccggcctggcctgtgacggtcagctgggtccc

SEQ ID NO: 14 - DNA, 38 bp, Artificial Sequence
  primer
actggccggcctggcctgaggagayrgtgaccagggtg

SEQ ID NO: 15 - DNA, 34 bp, Artificial Sequence
  primer
cgagctggagatcctaggtggttcctctagatct

SEQ ID NO: 16 - DNA, 34 bp, Artificial Sequence
  primer
caatgtggaaatcaaaggtggttcctctagatct

SEQ ID NO: 17 - DNA, 34 bp, Artificial Sequence
  primer
cgaggtggtsgtcaaaggtggttcctctagatct

SEQ ID NO: 18 - DNA, 28 bp, Artificial Sequence
  primer
actcctccaccgactgcccaccaccgcc

SEQ ID NO: 19 - DNA, 28 bp, Artificial Sequence
  primer
actccttcaccgactgcccaccaccgcc

SEQ ID NO: 20 - DNA, 28 bp, Artificial Sequence
  primer
actcctccarcgactgcccaccaccgcc

SEQ ID NO: 21 - DNA, 29 bp, Artificial Sequence
  primer
tccaycagctgctsctgcccaccaccgcc

SEQ ID NO: 22 - DNA, 38 bp, Artificial Sequence
  primer
gaggaggaggaggaggaggcggggcccaggcggccgag

SEQ ID NO: 23 - DNA, 38 bp, Artificial Sequence
  primer
gaggaggaggaggaggagcctggccggcctggcctgag

SEQ ID NO: 24 - protein, 116 aa, Artificial Sequence
  rabbit antibody 2-19 heavy chain variable region
QSVEESGGRLVTPGTPLTLTCTVSGIDLNRYSLTWVRQAPGKGLEWIGIVGGSGVTYYANWTKGRFTISKTSTTVDLKMTSLTTEDTATYFCARGSDRSAYAPDIWGPGTLVTISS

SEQ ID NO: 25 - protein, 112 aa, Artificial Sequence
  rabbit antibody 2-19 light chain variable region
ELDMTQTPSSVSAAVGGTVTINCQSSQSVYSNNYLAWYQQKPGQPPKLLLYQASKLASGVSSRFSGSGSGTHFTLTISGVQCDDAATYYCLGVYDDDADNAFGGGTELEILR

SEQ ID NO: 26 - DNA, 348 bp, Artificial Sequence
  rabbit antibody 2-19 heavy chain variable region
cagtcggtggaggagtccgggggtcgcctggtcacgcctgggacacccctgacactcacctgcacagtctctggaatcgacctcaataggtattcactgacctgggtccgccaggctccagggaaggggctggaatggatcggaatcgttggtggtagtggtgtcacatactacgcgaactggacgaaaggccgattcaccatctccaaaacctcgaccacggtggatctgaaaatgaccagtctgacaaccgaggacacggccacctatttctgtgccagaggatctgatcgtagtgcttatgcccctgacatctggggcccaggcaccctggtcaccatctcctca

SEQ ID NO: 27 - DNA, 336 bp, Artificial Sequence
  rabbit antibody 2-19 light chain variable region
gagctcgatatgacccagactccatcctccgtgtctgcagctgtgggaggcacagtcaccatcaattgccagtccagtcagagtgtttatagtaacaactacttagcctggtatcagcagaaaccagggcagcctcccaagctcctgctctaccaggcatccaaactggcatctggggtctcatcgcggttcagcggcagtggatctgggacacatttcactctcaccatcagcggcgtgcagtgtgacgatgctgccacttactactgtctaggcgtttatgatgatgatgctgataatgctttcggcggagggaccgagctggagatcctacgt

SEQ ID NO: 28 - protein, 119 aa, Artificial Sequence
  humanized antibody Hz1 HV
EVQLVESGGGLVKPGGSLRLSCAASGIDLNRYSLTWVRQAPGKGLEWVGIVGGSGVTYYANWAKGRFTISRDSAKNSLYLQMNSLRAEDTAVYFCARGSDRSAYAPDIWGPGTLVTVSS

SEQ ID NO: 29 - protein, 112 aa, Artificial Sequence
  humanized antibody Hz1 LV
DIQMTQSPSSLSASVGDRVTINCQSSQSIYSNNYLAWYQQKPGKPPKLLLYQASKLASGVPSRFSGSGSGTDFTLTISSLQPEDVATYYCLGVYDDDADNAFGGGTELEIKR

SEQ ID NO: 30 - protein, 119 aa, Artificial Sequence
  humanized antibody Hz2 HV
EVQLVESGGGLVQPGGSLRLSCAVSGIDLNRYSLTWIRQAPGKGLEWVAIVGGSGVTYYANWAKGRFTISRDDSKNTLYLQMNSLRAEDTAVYYCARGSDRSAYAPDIWGQGTLVTVSS

SEQ ID NO: 31 - protein, 112 aa, Artificial Sequence
  humanized antibody Hz2 LV
DIQLTQSPSSLSASVGDRVTITCQSSQSIYSNNYLAWYQQKPGKAPKLLLYQASKLASGVPSRFSGSGSGTDFTLTISSLQPEDFATYYCLGVYDDDADNAFGQGTKVEIKR

SEQ ID NO: 32 - protein, 123 aa, Artificial Sequence
  humanized antibody Lu007 HV
EVQLVESGGGLVQPGGSLRLSCAASGYDFTHYGMNWIRQAPGKGLEWVGWINTYTGEPTYAADFKRRFTFSLDTSKSTVYLQMNSLRAEDTAVYYCAKYPHYYGTSHWYFDVWGQGTLVTVSS

SEQ ID NO: 33 - protein, 108 aa, Artificial Sequence
  humanized antibody Lu007 LV
DIQLTQSPSSLSASVGDRVTITCSASQDISNYLNWYQQKPGKAPKVLIYFTSSLHSGVPSRFSGSGSGTDFTLTISSLQPEDFATYYCQQYSTVPWTFGQGTKVEIKR

SEQ ID NO: 34 - protein, 123 aa, Artificial Sequence
  humanized antibody F8 HV
EVQLVESGGGLVQPGGSLRLSCAASGYDFTHYGMNWIRQAPGKGLEWVGWINTYTGEPTYAADFKRRFTFSRDASKSTVYLQMNSLRAEDTAVYYCAKYPYYYGTSHWYFDVWGQGTLVTVSS

SEQ ID NO: 35 - protein, 123 aa, Artificial Sequence
  humanized antibody E9 HV
EVQLVESGGGLVQPGGSLRLSCAVSGYDFTHYGMNWIRQAPGKGLEWVGWINTYTGEPTYAADFKRRFTFSRDASKSTAYLQMNSLRAEDTAVYYCARYPYYYGTSHWYFDVWGQGTLVTVSS

SEQ ID NO: 36 - protein, 123 aa, Artificial Sequence
  humanized antibody H2 HV
EVQLVESGGGLVQPGGSLRLSCAVSGYDFTHYGMNWIRQAPGKGLEWVGWINTYTGEPTYAADFKRRFTFSRDASKSTAYLQMNSLRAEDTAVYYCAKYPYYYGTSHWYFDVWGQGTLVTVSS

SEQ ID NO: 37 - protein, 30 aa, Artificial Sequence
  humanized antibody Hz2 HFR1
EVQLVESGGGLVQPGGSLRLSCAVSGIDLN

SEQ ID NO: 38 - protein, 14 aa, Artificial Sequence
  humanized antibody Hz2 HFR2
WIRQAPGKGLEWVA

SEQ ID NO: 39 - protein, 32 aa, Artificial Sequence
  humanized antibody Hz2 HFR3
RFTISRDDSKNTLYLQMNSLRAEDTAVYYCAR

SEQ ID NO: 40 - protein, 11 aa, Artificial Sequence
  humanized antibody Hz2 or Lu007 HFR4
WGQGTLVTVSS

SEQ ID NO: 41 - protein, 23 aa, Artificial Sequence
  humanized antibody Hz2 or Lu007 LFR1
DIQLTQSPSSLSASVGDRVTITC

SEQ ID NO: 42 - protein, 15 aa, Artificial Sequence
  humanized antibody Hz2 LFR2
WYQQKPGKAPKLLLY

SEQ ID NO: 43 - protein, 32 aa, Artificial Sequence
  humanized antibody Hz2 or Lu007 LFR3
GVPSRFSGSGSGTDFTLTISSLQPEDFATYYC

SEQ ID NO: 44 - protein, 11 aa, Artificial Sequence
  humanized antibody Hz2 or Lu007 LFR4
FGQGTKVEIKR

SEQ ID NO: 45 - protein, 5 aa, Artificial Sequence
  humanized antibody Hz1 or Hz2 HCDR1
RYSLT

SEQ ID NO: 46 - protein, 16 aa, Artificial Sequence
  humanized antibody Hz1 or Hz2 HCDR2
IVGGSGVTYYANWAKG

SEQ ID NO: 47 - protein, 11 aa, Artificial Sequence
  humanized antibody Hz1 or Hz2 HCDR3
GSDRSAYAPDI

SEQ ID NO: 48 - protein, 13 aa, Artificial Sequence
  humanized antibody Hz1 or Hz2 LCDR1
QSSQSIYSNNYLA

SEQ ID NO: 49 - protein, 7 aa, Artificial Sequence
  humanized antibody Hz1 or Hz2 LCDR2
QASKLAS

SEQ ID NO: 50 - protein, 11 aa, Artificial Sequence
  humanized antibody Hz1 or Hz2 LCDR3
LGVYDDDADNA

SEQ ID NO: 51 - protein, 30 aa, Artificial Sequence
  humanized antibody Lu007 HFR1
EVQLVESGGGLVQPGGSLRLSCAASGYDFT

SEQ ID NO: 52 - protein, 14 aa, Artificial Sequence
  humanized antibody Lu007 HFR2
WIRQAPGKGLEWVG

SEQ ID NO: 53 - protein, 32 aa, Artificial Sequence
  humanized antibody Lu007 HFR3
RFTFSLDTSKSTVYLQMNSLRAEDTAVYYCAK

SEQ ID NO: 54 - protein, 15 aa, Artificial Sequence
  humanized antibody Lu007 LFR2
WYQQKPGKAPKVLIY

SEQ ID NO: 55 - protein, 5 aa, Artificial Sequence
  humanized antibody Lu007 HCDR1
HYGMN

SEQ ID NO: 56 - protein, 17 aa, Artificial Sequence
  humanized antibody Lu007 HCDR2
WINTYTGEPTYAADFKR

SEQ ID NO: 57 - protein, 14 aa, Artificial Sequence
  humanized antibody Lu007 HCDR3
YPHYYGTSHWYFDV

SEQ ID NO: 58 - protein, 11 aa, Artificial Sequence
  humanized antibody Lu007 LCDR1
SASQDISNYLN

SEQ ID NO: 59 - protein, 7 aa, Artificial Sequence
  humanized antibody Lu007 LCDR2
FTSSLHS

SEQ ID NO: 60 - protein, 9 aa, Artificial Sequence
  humanized antibody Lu007 LCDR3
QQYSTVPWT

SEQ ID NO: 61 - protein, 18 aa, Artificial Sequence
  mu-tailpiece
PTLYNVSLVMSDTAGTCY

SEQ ID NO: 62 - protein, 431 aa, Artificial Sequence
  AAA0289, Aflibercept
SDTGRPFVEMYSEIPEIIHMTEGRELVIPCRVTSPNITVTLKKFPLDTLIPDGKRIIWDSRKGFIISNATYKEIGLLTCEATVNGHLYKTNYLTHRQTNTIIDVVLSPSHGIELSVGEKLVLNCTARTELNVGIDFNWEYPSSKHQHKKLVNRDLKTQSGSEMKKFLSTLTIDGVTRSDQGLYTCAASSGLMTKKNSTFVRVHEKDKTHTCPPCPAPELLGGPSVFLFPPKPKDTLMISRTPEVTCVVVDVSHEDPEVKFNWYVDGVEVHNAKTKPREEQYNSTYRVVSVLTVLHQDWLNGKEYKCKVSNKALPAPIEKTISKAKGQPREPQVYTLPPSRDELTKNQVSLTCLVKGFYPSDIAVEWESNGQPENNYKTTPPVLDSDGSFFLYSKLTVDKSRWQQGNVFSCSVMHEALHNHYTQKSLSLSPG

SEQ ID NO: 63 - protein, 453 aa, Artificial Sequence
  AAA0292(Avastin) Heavy Chain
EVQLVESGGGLVQPGGSLRLSCAASGYTFTNYGMNWVRQAPGKGLEWVGWINTYTGEPTYAADFKRRFTFSLDTSKSTAYLQMNSLRAEDTAVYYCAKYPHYYGSSHWYFDVWGQGTLVTVSSASTKGPSVFPLAPSSKSTSGGTAALGCLVKDYFPEPVTVSWNSGALTSGVHTFPAVLQSSGLYSLSSVVTVPSSSLGTQTYICNVNHKPSNTKVDKKVEPKSCDKTHTCPPCPAPELLGGPSVFLFPPKPKDTLMISRTPEVTCVVVDVSHEDPEVKFNWYVDGVEVHNAKTKPREEQYNSTYRVVSVLTVLHQDWLNGKEYKCKVSNKALPAPIEKTISKAKGQPREPQVYTLPPSREEMTKNQVSLTCLVKGFYPSDIAVEWESNGQPENNYKTTPPVLDSDGSFFLYSKLTVDKSRWQQGNVFSCSVMHEALHNHYTQKSLSLSPGK

SEQ ID NO: 64 - protein, 214 aa, Artificial Sequence
  AAA0292(Avastin) Light Chain
DIQMTQSPSSLSASVGDRVTITCSASQDISNYLNWYQQKPGKAPKVLIYFTSSLHSGVPSRFSGSGSGTDFTLTISSLQPEDFATYYCQQYSTVPWTFGQGTKVEIKRTVAAPSVFIFPPSDEQLKSGTASVVCLLNNFYPREAKVQWKVDNALQSGNSQESVTEQDSKDSTYSLSSTLTLSKADYEKHKVYACEVTHQGLSSPVTKSFNRGEC

SEQ ID NO: 65 - protein, 471 aa, Artificial Sequence
  AAA0306(Avastin Hexamer) Heavy Chain
EVQLVESGGGLVQPGGSLRLSCAASGYTFTNYGMNWVRQAPGKGLEWVGWINTYTGEPTYAADFKRRFTFSLDTSKSTAYLQMNSLRAEDTAVYYCAKYPHYYGSSHWYFDVWGQGTLVTVSSASTKGPSVFPLAPSSKSTSGGTAALGCLVKDYFPEPVTVSWNSGALTSGVHTFPAVLQSSGLYSLSSVVTVPSSSLGTQTYICNVNHKPSNTKVDKKVEPKSCDKTHTCPPCPAPELLGGPSVFLFPPKPKDTLMISRTPEVTCVVVDVSHEDPEVKFNWYVDGVEVHNAKTKPREEQYNSTYRVVSVLTVCLQDWLNGKEYKCKVSNKALPAPIEKTISKAKGQPREPQVYTLPPSREEMTKNQVSLTCLVKGFYPSDIAVEWESNGQPENNYKTTPPVLDSDGSFFLYSKLTVDKSRWQQGNVFSCSVMHEALHNHYTQKSLSLSPGKPTLYNVSLVMSDTAGTCY

SEQ ID NO: 66 - protein, 450 aa, Artificial Sequence
  AAA0308(Aflibercept hexamer)
SDTGRPFVEMYSEIPEIIHMTEGRELVIPCRVTSPNITVTLKKFPLDTLIPDGKRIIWDSRKGFIISNATYKEIGLLTCEATVNGHLYKTNYLTHRQTNTIIDVVLSPSHGIELSVGEKLVLNCTARTELNVGIDFNWEYPSSKHQHKKLVNRDLKTQSGSEMKKFLSTLTIDGVTRSDQGLYTCAASSGLMTKKNSTFVRVHEKDKTHTCPPCPAPELLGGPSVFLFPPKPKDTLMISRTPEVTCVVVDVSHEDPEVKFNWYVDGVEVHNAKTKPREEQYNSTYRVVSVLTVCLQDWLNGKEYKCKVSNKALPAPIEKTISKAKGQPREPQVYTLPPSRDELTKNQVSLTCLVKGFYPSDIAVEWESNGQPENNYKTTPPVLDSDGSFFLYSKLTVDKSRWQQGNVFSCSVMHEALHNHYTQKSLSLSPGKPTLYNVSLVMSDTAGTCY

SEQ ID NO: 67 - protein, 467 aa, Artificial Sequence
  AAA0322(Hz1 hexamer) heavy chain
EVQLVESGGGLVKPGGSLRLSCAASGIDLNRYSLTWVRQAPGKCLEWVGIVGGSGVTYYANWAKGRFTISRDSAKNSLYLQMNSLRAEDTAVYFCARGSDRSAYAPDIWGPGTLVTVSSASTKGPSVFPLAPSSKSTSGGTAALGCLVKDYFPEPVTVSWNSGALTSGVHTFPAVLQSSGLYSLSSVVTVPSSSLGTQTYICNVNHKPSNTKVDKKVEPKSCDKTHTCPPCPAPELLGGPSVFLFPPKPKDTLMISRTPEVTCVVVDVSHEDPEVKFNWYVDGVEVHNAKTKPREEQYNSTYRVVSVLTVCLQDWLNGKEYKCKVSNKALPAPIEKTISKAKGQPREPQVYTLPPSREEMTKNQVSLTCLVKGFYPSDIAVEWESNGQPENNYKTTPPVLDSDGSFFLYSKLTVDKSRWQQGNVFSCSVMHEALHNHYTQKSLSLSPGKPTLYNVSLVMSDTAGTCY

SEQ ID NO: 68 - protein, 218 aa, Artificial Sequence
  AAA0322(Hz1 hexamer) light chain
DIQMTQSPSSLSASVGDRVTINCQSSQSIYSNNYLAWYQQKPGKPPKLLLYQASKLASGVPSRFSGSGSGTDFTLTISSLQPEDVATYYCLGVYDDDADNAFGCGTELEIKRTVAAPSVFIFPPSDEQLKSGTASVVCLLNNFYPREAKVQWKVDNALQSGNSQESVTEQDSKDSTYSLSSTLTLSKADYEKHKVYACEVTHQGLSSPVTKSFNRGEC

SEQ ID NO: 69 - protein, 467 aa, Artificial Sequence
  AAA0589(Hz2-F hexamer) heavy chain
EVQLVESGGGLVQPGGSLRLSCAVSGIDLNRYSLTWIRQAPGKGLEWVAIVGGSGVTYYANWAKGRFTISRDDSKNTLYLQMNSLRAEDTAVYYCARGSDRSAYAPDIWGQGTLVTVSSASTKGPSVFPLAPSSKSTSGGTAALGCLVKDYFPEPVTVSWNSGALTSGVHTFPAVLQSSGLYSLSSVVTVPSSSLGTQTYICNVNHKPSNTKVDKKVEPKSCDKTHTCPPCPAPEAAGGPSVFLFPPKPKDTLMISRTPEVTCVVVDVSHEDPEVKFNWYVDGVEVHNAKTKPREEQYNSTYRVVSVLTVCLQDWLNGKEYKCKVSNKALPAGIEKTISKAKGQPREPQVYTLPPSRDELTKNQVSLTCLVKGFYPSDIAVEWESNGQPENNYKTTPPVLDSDGSFFLYSKLTVDKSRWQQGNVFSCSVMHHALHNHYTQKSLSLSPGKPTLYNVSLVMSDTAGTCY

SEQ ID NO: 70 - protein, 218 aa, Artificial Sequence
  AAA0589(Hz2-F hexamer) light chain
DIQLTQSPSSLSASVGDRVTITCQSSQSIYSNNYLAWYQQKPGKAPKLLLYQASKLASGVPSRFSGSGSGTDFTLTISSLQPEDFATYYCLGVYDDDADNAFGQGTKVEIKRTVAAPSVFIFPPSDEQLKSGTASVVCLLNNFYPREAKVQWKVDNALQSGNSQESVTEQDSKDSTYSLSSTLTLSKADYEKHKVYACEVTHQGLSSPVTKSFNRGEC

SEQ ID NO: 71 - protein, 471 aa, Artificial Sequence
  AAA0592(Lu007-F hexamer) heavy chain
EVQLVESGGGLVQPGGSLRLSCAASGYDFTHYGMNWIRQAPGKGLEWVGWINTYTGEPTYAADFKRRFTFSLDTSKSTVYLQMNSLRAEDTAVYYCAKYPHYYGTSHWYFDVWGQGTLVTVSSASTKGPSVFPLAPSSKSTSGGTAALGCLVKDYFPEPVTVSWNSGALTSGVHTFPAVLQSSGLYSLSSVVTVPSSSLGTQTYICNVNHKPSNTKVDKKVEPKSCDKTHTCPPCPAPEAAGGPSVFLFPPKPKDTLMISRTPEVTCVVVDVSHEDPEVKFNWYVDGVEVHNAKTKPREEQYNSTYRVVSVLTVCLQDWLNGKEYKCKVSNKALPAGIEKTISKAKGQPREPQVYTLPPSRDELTKNQVSLTCLVKGFYPSDIAVEWESNGQPENNYKTTPPVLDSDGSFFLYSKLTVDKSRWQQGNVFSCSVMHEALHNHYTQKSLSLSPGKPTLYNVSLVMSDTAGTCY

SEQ ID NO: 72 - protein, 214 aa, Artificial Sequence
  AAA0592(Lu007-F hexamer) light chain
DIQLTQSPSSLSASVGDRVTITCSASQDISNYLNWYQQKPGKAPKVLIYFTSSLHSGVPSRFSGSGSGTDFTLTISSLQPEDFATYYCQQYSTVPWTFGQGTKVEIKRTVAAPSVFIFPPSDEQLKSGTASVVCLLNNFYPREAKVQWKVDNALQSGNSQESVTEQDSKDSTYSLSSTLTLSKADYEKHKVYACEVTHQGLSSPVTKSFNRGEC

SEQ ID NO: 73 - protein, 562 aa, Artificial Sequence
  AAA0600(Aflibercept CL kappa hexamer)
SDTGRPFVEMYSEIPEIIHMTEGRELVIPCRVTSPNITVTLKKFPLDTLIPDGKRIIWDSRKGFIISNATYKEIGLLTCEATVNGHLYKTNYLTHRQTNTIIDVVLSPSHGIELSVGEKLVLNCTARTELNVGIDFNWEYPSSKHQHKKLVNRDLKTQSGSEMKKFLSTLTIDGVTRSDQGLYTCAASSGLMTKKNSTFVRVHEKTVAAPRTVAAPSVFIFPPSDEQLKSGTASVVCLLNNFYPREAKVQWKVDNALQSGNSQESVTEQDSKDSTYSLSSTLTLSKADYEKHKVYACEVTHQGLSSPVTKSFNRGESDKTHTCPPCPAPEAAGGPSVFLFPPKPKDTLMISRTPEVTCVVVDVSHEDPEVKFNWYVDGVEVHNAKTKPREEQYNSTYRVVSVLTVCLQDWLNGKEYKCKVSNKALPAGIEKTISKAKGQPREPQVYTLPPSRDELTKNQVSLTCLVKGFYPSDIAVEWESNGQPENNYKTTPPVLDSDGSFFLYSKLTVDKSRWQQGNVFSCSVMHHALHNHYTQKSLSLSPGKPTLYNVSLVMSDTAGTCY

SEQ ID NO: 74 - protein, 227 aa, Artificial Sequence
  AAA0589(Hz2-F hexamer) heavy chain Fc region
DKTHTCPPCPAPEAAGGPSVFLFPPKPKDTLMISRTPEVTCVVVDVSHEDPEVKFNWYVDGVEVHNAKTKPREEQYNSTYRVVSVLTVCLQDWLNGKEYKCKVSNKALPAGIEKTISKAKGQPREPQVYTLPPSRDELTKNQVSLTCLVKGFYPSDIAVEWESNGQPENNYKTTPPVLDSDGSFFLYSKLTVDKSRWQQGNVFSCSVMHHALHNHYTQKSLSLSPGK

SEQ ID NO: 75 - protein, 227 aa, Artificial Sequence
  AAA0592(Lu007-F hexamer) heavy chain Fc region
DKTHTCPPCPAPEAAGGPSVFLFPPKPKDTLMISRTPEVTCVVVDVSHEDPEVKFNWYVDGVEVHNAKTKPREEQYNSTYRVVSVLTVCLQDWLNGKEYKCKVSNKALPAGIEKTISKAKGQPREPQVYTLPPSRDELTKNQVSLTCLVKGFYPSDIAVEWESNGQPENNYKTTPPVLDSDGSFFLYSKLTVDKSRWQQGNVFSCSVMHEALHNHYTQKSLSLSPGK

SEQ ID NO: 76 - protein, 449 aa, Artificial Sequence
  Omal013 heavy chain
EVQLVESGGGLVQPGGSLRLSCAVSGIDLNRYSLTWIRQAPGKGLEWVAIVGGSGVTYYANWAKGRFTISRDDSKNTLYLQMNSLRAEDTAVYYCARGSDRSAYAPDIWGQGTLVTVSSASTKGPSVFPLAPSSKSTSGGTAALGCLVKDYFPEPVTVSWNSGALTSGVHTFPAVLQSSGLYSLSSVVTVPSSSLGTQTYICNVNHKPSNTKVDKKVEPKSCDKTHTCPPCPAPELLGGPSVFLFPPKPKDTLMISRTPEVTCVVVDVSHEDPEVKFNWYVDGVEVHNAKTKPREEQYNSTYRVVSVLTVLHQDWLNGKEYKCKVSNKALPAPIEKTISKAKGQPREPQVYTLPPSRDELTKNQVSLTCLVKGFYPSDIAVEWESNGQPENNYKTTPPVLDSDGSFFLYSKLTVDKSRWQQGNVFSCSVMHEALHNHYTQKSLSLSPGK